European Patent Application EP 4 140 302 A1, published March 1, 2023. Title: Use of (Z)-3-hexenyl esters and method to protect plants against pests. Applicant: Universitat Politècnica de València (UPV) Instituto Valenciano de Investigaciones Agrarias (IVIA) Consejo Superior de Investigaciones Científicas (CSIC). The sequence listing filed with the application follows.

SEQUENCE LISTING (18 sequences)

SEQ ID NO: 1 - DNA, 21 bp, Artificial Sequence
  Forward primer PR1
ctcatatgagacgtcgagaag

SEQ ID NO: 2 - DNA, 25 bp, Artificial Sequence
  Reverse primer PR1
ggaaacaagaagatgcagtacttaa

SEQ ID NO: 3 - DNA, 20 bp, Artificial Sequence
  Forward primer Sl-PI-I
tgaaactctcatggcacgaa

SEQ ID NO: 4 - DNA, 22 bp, Artificial Sequence
  Reverse primer Sl-PI-I
ttttgacatattgtggctgctt

SEQ ID NO: 5 - DNA, 20 bp, Artificial Sequence
  Forward primer Sl-PI-II
ggccaaatgcttgcaccttt

SEQ ID NO: 6 - DNA, 20 bp, Artificial Sequence
  Reverse primer Sl-PI-II
caacacgtggtacatccggt

SEQ ID NO: 7 - DNA, 22 bp, Artificial Sequence
  Forward primer EF1
gattggtggtattggaactgtc

SEQ ID NO: 8 - DNA, 18 bp, Artificial Sequence
  Reverse primer EF1
agcttcgtggtgcatctc

SEQ ID NO: 9 - DNA, 22 bp, Artificial Sequence
  Forward primer PIN2
gaaaatcgttaatttatcccac

SEQ ID NO: 10 - DNA, 22 bp, Artificial Sequence
  Reverse primer PIN2
acatacaaactttccatcttta

SEQ ID NO: 11 - DNA, 20 bp, Artificial Sequence
  Forward primer LOX2
gaaccatattgccactttcg

SEQ ID NO: 12 - DNA, 20 bp, Artificial Sequence
  Reverse primer LOX2
cgtcatcaatgacttgacca

SEQ ID NO: 13 - DNA, 21 bp, Artificial Sequence
  Forward primer PAL
cacattcttggtagcgctttg

SEQ ID NO: 14 - DNA, 22 bp, Artificial Sequence
  Reverse primer PAL
agctacttggctgacagtattc

SEQ ID NO: 15 - DNA, 22 bp, Artificial Sequence
  Forward primer NPR5
tacctccacctctctcattctt

SEQ ID NO: 16 - DNA, 22 bp, Artificial Sequence
  Reverse primer NPR5
gtgcgagagaaggttagctatg

SEQ ID NO: 17 - DNA, 22 bp, Artificial Sequence
  Forward primer GAPDH
ggaaggtcaagatcggaatcaa

SEQ ID NO: 18 - DNA, 22 bp, Artificial Sequence
  Reverse primer GAPDH
cgtccctctgcaagatgactct